European Patent Application EP 4 227 322 A1, published August 16, 2023. Title: ANTIBODIES TARGETING THE B-CELL RECEPTOR OF CHRONIC LYMPHOCYTIC LEUKEMIA AND USES THEREOF. Applicant: AVA Lifescience GmbH. The sequence listing filed with the application follows.

SEQUENCE LISTING (53 sequences)

SEQ ID NO: 1 - protein, 443 aa, Mus musculus
QVQLQQSGPGLVQPSQSLSITCTVSGFSLTSYGIHWVRQSPGKGLEWLGVIWRGGGTDSNAAFMSRLSITKDNSKSQVFFKMNSLQADDTAIYYCARSRYDEEESMNYWGQGTSVTVSSAKTTPPSVYPLAPGSAAQTNSMVTLGCLVKGYFPEPVTVTWNSGSLSSGVHTFPAVLQSDLYTLSSSVTVPSSPRPSETVTCNVAHPASSTKVDKKIVPRDCGCKPCICTVPEVSSVFIFPPKPKDVLTITLTPKVTCVVVDISKDDPEVQFSWFVDDVEVHTAQTQPREEQFNSTFRSVSELPIMHQDWLNGKEFKCRVNSAAFPAPIEKTISKTKGRPKAPQVYTIPPPKEQMAKDKVSLTCMITDFFPEDITVEWQWNGQPAENYKNTQPIMNTNGSYFVYSKLNVQKSNWEAGNTFTCSVLHEGLHNHHTEKSLSHSPGK

SEQ ID NO: 2 - protein, 214 aa, Mus musculus
QIVLTQSPASLSASVGETVTITCRASGNIHSYLAWYQQKQGKSPQLLVYNAKTLADGVPSRFSGSGSGTQYSLKINSLQPEDFGSYYCQHFWNTPPTFGAGTKLELKRADAAPTVSIFPPSSEQLTSGGASVVCFLNNFYPKDINVKWKIDGSERQNGVLNSWTDQDSKDSTYSMSSTLTLTKDEYERHNSYTCEATHKTSTSPIVKSFNRNEC

SEQ ID NO: 3 - protein, 119 aa, Mus musculus
QVQLQQSGPGLVQPSQSLSITCTVSGFSLTSYGIHWVRQSPGKGLEWLGVIWRGGGTDSNAAFMSRLSITKDNSKSQVFFKMNSLQADDTAIYYCARSRYDEEESMNYWGQGTSVTVSS

SEQ ID NO: 4 - protein, 108 aa, Mus musculus
QIVLTQSPASLSASVGETVTITCRASGNIHSYLAWYQQKQGKSPQLLVYNAKTLADGVPSRFSGSGSGTQYSLKINSLQPEDFGSYYCQHFWNTPPTFGAGTKLELKR

SEQ ID NO: 5 - protein, 8 aa, Mus musculus
GFSLTSYG

SEQ ID NO: 6 - protein, 7 aa, Mus musculus
IWRGGGT

SEQ ID NO: 7 - protein, 13 aa, Mus musculus
ARSRYDEEESMNY

SEQ ID NO: 8 - protein, 6 aa, Mus musculus
GNIHSY

SEQ ID NO: 9 - protein, 4 aa, Mus musculus
NAKT

SEQ ID NO: 10 - protein, 9 aa, Mus musculus
QHFWNTPPT

SEQ ID NO: 11 - protein, 449 aa, synthetic construct
QVQLQQSGPGLVQPSQSLSITCTVSGFSLTSYGIHWVRQSPGKGLEWLGVIWRGGGTDSNAAFMSRLSITKDNSKSQVFFKMNSLQADDTAIYYCARSRYDEEESMNYWGQGTSVTVSSASTKGPSVFPLAPSSKSTSGGTAALGCLVKDYFPEPVTVSWNSGALTSGVHTFPAVLQSSGLYSLSSVVTVPSSSLGTQTYICNVNHKPSNTKVDKKVEPKSCDKTHTCPPCPAPELLGGPSVFLFPPKPKDTLMISRTPEVTCVVVDVSHEDPEVKFNWYVDGVEVHNAKTKPREEQYNSTYRVVSVLTVLHQDWLNGKEYKCKVSNKALPAPIEKTISKAKGQPREPQVYTLPPSRDELTKNQVSLTCLVKGFYPSDIAVEWESNGQPENNYKTTPPVLDSDGSFFLYSKLTVDKSRWQQGNVFSCSVMHEALHNHYTQKSLSLSPGK

SEQ ID NO: 12 - protein, 214 aa, synthetic construct
QIVLTQSPASLSASVGETVTITCRASGNIHSYLAWYQQKQGKSPQLLVYNAKTLADGVPSRFSGSGSGTQYSLKINSLQPEDFGSYYCQHFWNTPPTFGAGTKLELKRTVAAPSVFIFPPSDEQLKSGTASVVCLLNNFYPREAKVQWKVDNALQSGNSQESVTEQDSKDSTYSLSSTLTLSKADYEKHKVYACEVTHQGLSSPVTKSFNRGEC

SEQ ID NO: 13 - protein, 449 aa, synthetic construct
QVQLQESGPGLVKPSETLSLTCTVSGFSLTSYGIHWIRQSPGRGLEWIGVIWRGGGTDSNAAFMSRITISRDTSKTQVSLKLGSVTAADTAIYYCARSRYDEEESMNYWGQGTSVTVSSASTKGPSVFPLAPSSKSTSGGTAALGCLVKDYFPEPVTVSWNSGALTSGVHTFPAVLQSSGLYSLSSVVTVPSSSLGTQTYICNVNHKPSNTKVDKKVEPKSCDKTHTCPPCPAPELLGGPSVFLFPPKPKDTLMISRTPEVTCVVVDVSHEDPEVKFNWYVDGVEVHNAKTKPREEQYNSTYRVVSVLTVLHQDWLNGKEYKCKVSNKALPAPIEKTISKAKGQPREPQVYTLPPSRDELTKNQVSLTCLVKGFYPSDIAVEWESNGQPENNYKTTPPVLDSDGSFFLYSKLTVDKSRWQQGNVFSCSVMHEALHNHYTQKSLSLSPGK

SEQ ID NO: 14 - protein, 214 aa, synthetic construct
EIVLTQSPSSLSASVGDSVTITCRASGNIHSYLAWYQQKPGKAPKLLIYNAKTLADGVPSRFSGSGSGTQYTLTISSLQPEDFATYYCQHFWNTPPTFGAGTKLELKRTVAAPSVFIFPPSDEQLKSGTASVVCLLNNFYPREAKVQWKVDNALQSGNSQESVTEQDSKDSTYSLSSTLTLSKADYEKHKVYACEVTHQGLSSPVTKSFNRGEC

SEQ ID NO: 15 - protein, 119 aa, synthetic construct
QVQLQESGPGLVKPSETLSLTCTVSGFSLTSYGIHWIRQSPGRGLEWIGVIWRGGGTDSNAAFMSRITISRDTSKTQVSLKLGSVTAADTAIYYCARSRYDEEESMNYWGQGTSVTVSS

SEQ ID NO: 16 - protein, 108 aa, synthetic construct
EIVLTQSPSSLSASVGDSVTITCRASGNIHSYLAWYQQKPGKAPKLLIYNAKTLADGVPSRFSGSGSGTQYTLTISSLQPEDFATYYCQHFWNTPPTFGAGTKLELKR

SEQ ID NO: 17 - protein, 108 aa, synthetic construct
QIQLTQSPSFLSASVGDSVTITCRASGNIHSYLAWYQQKPGKAPQLLIYNAKTLADGVPSRFSGSGSGTEYTLTISSLQPEDFATYYCQHFWNTPPTFGAGTKLELKR

SEQ ID NO: 18 - protein, 108 aa, synthetic construct
EIVLTQSPATLSLSPGERATLSCRASGNIHSYLAWYQQKPGQAPRLLIYNAKTLADGIPARFSGSGSGTDYTLTISSLEPEDFASYYCQHFWNTPPTFGAGTKLELKR

SEQ ID NO: 19 - protein, 108 aa, synthetic construct
EIVLTQSPGTLSLSPGERATLSCRASGNIHSYLAWYQQKPGQAPRLLIYNAKTLADGIPDRFSGSGSGTDYTLTISRLEPEDFAVYYCQHFWNTPPTFGAGTKLELKR

SEQ ID NO: 20 - protein, 119 aa, synthetic construct; identical to SEQ ID NO: 15

SEQ ID NO: 21 - protein, 449 aa, synthetic construct; identical to SEQ ID NO: 13

SEQ ID NO: 22 - protein, 214 aa, synthetic construct
QIQLTQSPSFLSASVGDSVTITCRASGNIHSYLAWYQQKPGKAPQLLIYNAKTLADGVPSRFSGSGSGTEYTLTISSLQPEDFATYYCQHFWNTPPTFGAGTKLELKRTVAAPSVFIFPPSDEQLKSGTASVVCLLNNFYPREAKVQWKVDNALQSGNSQESVTEQDSKDSTYSLSSTLTLSKADYEKHKVYACEVTHQGLSSPVTKSFNRGEC

SEQ ID NO: 23 - protein, 214 aa, synthetic construct
EIVLTQSPATLSLSPGERATLSCRASGNIHSYLAWYQQKPGQAPRLLIYNAKTLADGIPARFSGSGSGTDYTLTISSLEPEDFASYYCQHFWNTPPTFGAGTKLELKRTVAAPSVFIFPPSDEQLKSGTASVVCLLNNFYPREAKVQWKVDNALQSGNSQESVTEQDSKDSTYSLSSTLTLSKADYEKHKVYACEVTHQGLSSPVTKSFNRGEC

SEQ ID NO: 24 - protein, 214 aa, synthetic construct
EIVLTQSPGTLSLSPGERATLSCRASGNIHSYLAWYQQKPGQAPRLLIYNAKTLADGIPDRFSGSGSGTDYTLTISRLEPEDFAVYYCQHFWNTPPTFGAGTKLELKRTVAAPSVFIFPPSDEQLKSGTASVVCLLNNFYPREAKVQWKVDNALQSGNSQESVTEQDSKDSTYSLSSTLTLSKADYEKHKVYACEVTHQGLSSPVTKSFNRGEC

SEQ ID NO: 25 - DNA, 1329 bp, synthetic construct
  source 1..1329: mol_type = other DNA
caggtgcagctgcagcagtctggacctggcctagtgcagccctcacagagcctgtccataacctgcacagtctctggtttctcattaactagctatggtatacactgggttcgccagtctccaggaaagggtctggagtggctgggagtgatatggagaggtggaggcacagactccaatgcagctttcatgtccagactgagcatcaccaaggacaattccaagagccaagttttctttaaaatgaacagtctgcaagctgatgacactgccatatattactgtgccagaagtaggtacgacgaggaggaaagtatgaactactggggtcaaggaacctcagtcaccgtctcctcagccaaaacgacacccccatctgtctatccactggcccctggatctgctgcccaaactaactccatggtgaccctgggatgcctggtcaagggctatttccctgagccagtgacagtgacctggaactctggatccctgtccagcggtgtgcacaccttcccagctgtcctgcagtctgacctctacactctgagcagctcagtgactgtcccctccagccctcggcccagcgagaccgtcacctgcaacgttgcccacccggccagcagcaccaaggtggacaagaaaattgtgcccagggattgtggttgtaagccttgcatatgtacagtcccagaagtatcatctgtcttcatcttccccccaaagcccaaggatgtgctcaccattactctgactcctaaggtcacgtgtgttgtggtagacatcagcaaggatgatcccgaggtccagttcagctggtttgtagatgatgtggaggtgcacacagctcagacgcaaccccgggaggagcagttcaacagcactttccgctcagtcagtgaacttcccatcatgcaccaggactggctcaatggcaaggagttcaaatgcagggtcaacagtgcagctttccctgcccccatcgagaaaaccatctccaaaaccaaaggcagaccgaaggctccacaggtgtacaccattccacctcccaaggagcagatggccaaggataaagtcagtctgacctgcatgataacagacttcttccctgaagacattactgtggagtggcagtggaatgggcagccagcggagaactacaagaacactcagcccatcatgaacacgaatggctcttacttcgtctacagcaagctcaatgtgcagaagagcaactgggaggcaggaaatactttcacctgctctgtgttacatgagggcctgcacaaccaccatactgagaagagcctctcccactctcctggtaaa

SEQ ID NO: 26 - DNA, 642 bp, synthetic construct
  source 1..642: mol_type = other DNA
caaattgttctcacccagtctccagcctccctatctgcatctgtgggagaaactgtcaccatcacttgtcgagcaagtgggaatattcacagttatttagcatggtatcagcagaaacagggaaaatctcctcagctcctggtctataatgcaaaaaccttagcagatggtgtgccatcaaggttcagtggcagtggatcaggaacacaatattctctcaagatcaacagcctgcagcctgaagattttgggagttattactgtcaacatttttggaatactcctcccacgttcggtgctgggaccaagctggagctgaaacgggctgatgctgcaccaactgtatccatcttcccaccatccagtgagcagttaacatctggaggtgcctcagtcgtgtgcttcttgaacaacttctaccccaaagacatcaatgtcaagtggaagattgatggcagtgaacgacaaaatggcgtcctgaacagttggactgatcaggacagcaaagacagcacctacagcatgagcagcaccctcacgttgaccaaggacgagtatgaacgacataacagctatacctgtgaggccactcacaagacatcaacttcacccattgtcaagagcttcaacaggaatgagtgt

SEQ ID NO: 27 - DNA, 357 bp, synthetic construct
  source 1..357: mol_type = other DNA
caggtgcagctgcagcagtctggacctggcctagtgcagccctcacagagcctgtccataacctgcacagtctctggtttctcattaactagctatggtatacactgggttcgccagtctccaggaaagggtctggagtggctgggagtgatatggagaggtggaggcacagactccaatgcagctttcatgtccagactgagcatcaccaaggacaattccaagagccaagttttctttaaaatgaacagtctgcaagctgatgacactgccatatattactgtgccagaagtaggtacgacgaggaggaaagtatgaactactggggtcaaggaacctcagtcaccgtctcctca

SEQ ID NO: 28 - DNA, 321 bp, synthetic construct
  source 1..321: mol_type = other DNA
caaattgttctcacccagtctccagcctccctatctgcatctgtgggagaaactgtcaccatcacttgtcgagcaagtgggaatattcacagttatttagcatggtatcagcagaaacagggaaaatctcctcagctcctggtctataatgcaaaaaccttagcagatggtgtgccatcaaggttcagtggcagtggatcaggaacacaatattctctcaagatcaacagcctgcagcctgaagattttgggagttattactgtcaacatttttggaatactcctcccacgttcggtgctgggaccaagctggagctgaaa

SEQ ID NO: 29 - DNA, 1347 bp, synthetic construct
  source 1..1347: mol_type = other DNA
caggtgcagctgcagcagtctggacctggcctagtgcagccctcacagagcctgtccataacctgcacagtctctggtttctcattaactagctatggtatacactgggttcgccagtctccaggaaagggtctggagtggctgggagtgatatggagaggtggaggcacagactccaatgcagctttcatgtccagactgagcatcaccaaggacaattccaagagccaagttttctttaaaatgaacagtctgcaagctgatgacactgccatatattactgtgccagaagtaggtacgacgaggaggaaagtatgaactactggggtcaaggaacctcagtcaccgtctcctcagccagcaccaagggccccagcgtgttccccctggcccccagcagcaagagcaccagcggcggcaccgccgccctgggctgcctggtgaaggactacttccccgagcccgtgaccgtgagctggaacagcggcgccctgaccagcggcgtgcacaccttccccgccgtgctgcagagcagcggcctgtacagcctgagcagcgtggtgaccgtgcccagcagcagcctgggcacccagacctacatctgcaacgtgaaccacaagcccagcaacaccaaggtggacaagaaggtggagcccaagagctgcgacaagacccacacctgccccccctgccccgcccccgagctgctgggcggccccagcgtgttcctgttcccccccaagcccaaggacaccctgatgatcagcaggacccccgaggtgacctgcgtggtggtggacgtgagccacgaggaccccgaggtgaagttcaactggtacgtggacggcgtggaggtgcacaacgccaagaccaagcccagggaggagcagtacaacagcacctacagggtggtgagcgtgctgaccgtgctgcaccaggactggctgaacggcaaggagtacaagtgcaaggtgagcaacaaggccctgcccgcccccatcgagaagaccatcagcaaggccaagggccagcccagggagccccaggtgtacaccctgccccccagcagggacgagctgaccaagaaccaggtgagcctgacctgcctggtgaagggcttctaccccagcgacatcgccgtggagtgggagagcaacggccagcccgagaacaactacaagaccaccccccccgtgctggacagcgacggcagcttcttcctgtacagcaagctgaccgtggacaagagcaggtggcagcagggcaacgtgttcagctgcagcgtgatgcacgaggccctgcacaaccactacacccagaagagcctgagcctgagccccggcaag

SEQ ID NO: 30 - DNA, 642 bp, synthetic construct
  source 1..642: mol_type = other DNA
caaattgttctcacccagtctccagcctccctatctgcatctgtgggagaaactgtcaccatcacttgtcgagcaagtgggaatattcacagttatttagcatggtatcagcagaaacagggaaaatctcctcagctcctggtctataatgcaaaaaccttagcagatggtgtgccatcaaggttcagtggcagtggatcaggaacacaatattctctcaagatcaacagcctgcagcctgaagattttgggagttattactgtcaacatttttggaatactcctcccacgttcggtgctgggaccaagctggagctgaaacgcaccgtggcggcgccgagcgtgtttatttttccgccgagcgatgaacagctgaaaagcggcaccgcgagcgtggtgtgcctgctgaacaacttttatccgcgcgaagcgaaagtgcagtggaaagtggataacgcgctgcagagcggcaacagccaggaaagcgtgaccgaacaggatagcaaagatagcacctatagcctgagcagcaccctgaccctgagcaaagcggattatgaaaaacataaagtgtatgcgtgcgaagtgacccatcagggcctgagcagcccggtgaccaaaagctttaaccgcggcgaatgc

SEQ ID NO: 31 - DNA, 990 bp, synthetic construct
  source 1..990: mol_type = other DNA
gccagcaccaagggccccagcgtgttccccctggcccccagcagcaagagcaccagcggcggcaccgccgccctgggctgcctggtgaaggactacttccccgagcccgtgaccgtgagctggaacagcggcgccctgaccagcggcgtgcacaccttccccgccgtgctgcagagcagcggcctgtacagcctgagcagcgtggtgaccgtgcccagcagcagcctgggcacccagacctacatctgcaacgtgaaccacaagcccagcaacaccaaggtggacaagaaggtggagcccaagagctgcgacaagacccacacctgccccccctgccccgcccccgagctgctgggcggccccagcgtgttcctgttcccccccaagcccaaggacaccctgatgatcagcaggacccccgaggtgacctgcgtggtggtggacgtgagccacgaggaccccgaggtgaagttcaactggtacgtggacggcgtggaggtgcacaacgccaagaccaagcccagggaggagcagtacaacagcacctacagggtggtgagcgtgctgaccgtgctgcaccaggactggctgaacggcaaggagtacaagtgcaaggtgagcaacaaggccctgcccgcccccatcgagaagaccatcagcaaggccaagggccagcccagggagccccaggtgtacaccctgccccccagcagggacgagctgaccaagaaccaggtgagcctgacctgcctggtgaagggcttctaccccagcgacatcgccgtggagtgggagagcaacggccagcccgagaacaactacaagaccaccccccccgtgctggacagcgacggcagcttcttcctgtacagcaagctgaccgtggacaagagcaggtggcagcagggcaacgtgttcagctgcagcgtgatgcacgaggccctgcacaaccactacacccagaagagcctgagcctgagccccggcaag

SEQ ID NO: 32 - DNA, 321 bp, synthetic construct
  source 1..321: mol_type = other DNA
cgcaccgtggcggcgccgagcgtgtttatttttccgccgagcgatgaacagctgaaaagcggcaccgcgagcgtggtgtgcctgctgaacaacttttatccgcgcgaagcgaaagtgcagtggaaagtggataacgcgctgcagagcggcaacagccaggaaagcgtgaccgaacaggatagcaaagatagcacctatagcctgagcagcaccctgaccctgagcaaagcggattatgaaaaacataaagtgtatgcgtgcgaagtgacccatcagggcctgagcagcccggtgaccaaaagctttaaccgcggcgaatgc

SEQ ID NO: 33 - DNA, 357 bp, synthetic construct
  source 1..357: mol_type = other DNA
caggtgcagctgcaggagagcggccccggcctggtgaagcccagcgagaccctgagcctgacctgcaccgtgagcggcttcagcctgaccagctacggcatccactggatcaggcagagccccggcaggggcctggagtggatcggcgtgatctggaggggcggcggcaccgacagcaacgccgccttcatgagcagggtgaccatcagcagggacaccagcaagagccaggtgagcctgaagctgggcagcgtgaccgccgccgacaccgccatctactactgcgccaggagcaggtacgacgaggaggagagcatgaactactggggccagggcaccagcgtgaccgtgagcagc

SEQ ID NO: 34 - DNA, 321 bp, synthetic construct
  source 1..321: mol_type = other DNA
gaaattgtgctgacccagagcccgagcagcctgagcgcgagcgtgggcgatagcgtgaccattacctgccgcgcgagcggcaacattcatagctatctggcgtggtatcagcagaaaccgggcaaagcgccgaaactgctgatttataacgcgaaaaccctggcggatggcgtgccgagccgctttagcggcagcggcagcggcacccagtataccctgaccattagcagcctgcagccggaagattttgcgacctattattgccagcatttttggaacaccccgccgacctttggcgcgggcaccaaactggaactgaaa

SEQ ID NO: 35 - DNA, 321 bp, synthetic construct
  source 1..321: mol_type = other DNA
cagattcagctgacccagagcccgagctttctgagcgcgagcgtgggcgatagcgtgaccattacctgccgcgcgagcggcaacattcatagctatctggcgtggtatcagcagaaaccgggcaaagcgccgcagctgctgatttataacgcgaaaaccctggcggatggcgtgccgagccgctttagcggcagcggcagcggcaccgaatataccctgaccattagcagcctgcagccggaagattttgcgacctattattgccagcatttttggaacaccccgccgacctttggcgcgggcaccaaactggaactgaaa

SEQ ID NO: 36 - DNA, 321 bp, synthetic construct
  source 1..321: mol_type = other DNA
gagatcgtgctgacccagagccccgccaccctgagcctgagccccggcgagagggccaccctgagctgcagggccagcggcaacatccacagctacctggcctggtaccagcagaagcccggccaggcccccaggctgctgatctacaacgccaagaccctggccgacggcatccccgccaggttcagcggcagcggcagcggcaccgactacaccctgaccatcagcagcctggagcccgaggacttcgccagctactactgccagcacttctggaacaccccccccaccttcggcgccggcaccaagctggagctgaag

SEQ ID NO: 37 - DNA, 321 bp, synthetic construct
  source 1..321: mol_type = other DNA
gagatcgtgctgacccagagccccggcaccctgagcctgagccccggcgagagggccaccctgagctgcagggccagcggcaacatccacagctacctggcctggtaccagcagaagcccggccaggcccccaggctgctgatctacaacgccaagaccctggccgacggcatccccgacaggttcagcggcagcggcagcggcaccgactacaccctgaccatcagcaggctggagcccgaggacttcgccgtgtactactgccagcacttctggaacaccccccccaccttcggcgccggcaccaagctggagctgaag

SEQ ID NO: 38 - DNA, 357 bp, synthetic construct
  source 1..357: mol_type = other DNA
caggtgcagctgcaggagagcggccccggcctggtgaagcccagcgagaccctgagcctgacctgcaccgtgagcggcttcagcctgaccagctacggcatccactggatcaggcagagccccggcaggggcctggagtggatcggcgtgatctggaggggcggcggcaccgacagcaacgccgccttcatgagcaggatcaccatcagcagggacaccagcaagacccaggtgagcctgaagctgggcagcgtgaccgccgccgacaccgccatctactactgcgccaggagcaggtacgacgaggaggagagcatgaactactggggccagggcaccagcgtgaccgtgagcagc

SEQ ID NO: 39 - protein, 657 aa, synthetic construct
QVQLQQSGPGLVQPSQSLSITCTVSGFSLTSYGIHWVRQSPGKGLEWLGVIWRGGGTDSNAAFMSRLSITKDNSKSQVFFKMNSLQADDTAIYYCARSRYDEEESMNYWGQGTSVTVSSAKTTPPSVYPLAPGSAAQTNSMVTLGCLVKGYFPEPVTVTWNSGSLSSGVHTFPAVLQSDLYTLSSSVTVPSSPRPSETVTCNVAHPASSTKVDKKIVPRDCGCKPCICTVPEVSSVFIFPPKPKDVLTITLTPKVTCVVVDISKDDPEVQFSWFVDDVEVHTAQTQPREEQFNSTFRSVSELPIMHQDWLNGKEFKCRVNSAAFPAPIEKTISKTKGRPKAPQVYTIPPPKEQMAKDKVSLTCMITDFFPEDITVEWQWNGQPAENYKNTQPIMNTNGSYFVYSKLNVQKSNWEAGNTFTCSVLHEGLHNHHTEKSLSHSPGKQIVLTQSPASLSASVGETVTITCRASGNIHSYLAWYQQKQGKSPQLLVYNAKTLADGVPSRFSGSGSGTQYSLKINSLQPEDFGSYYCQHFWNTPPTFGAGTKLELKRADAAPTVSIFPPSSEQLTSGGASVVCFLNNFYPKDINVKWKIDGSERQNGVLNSWTDQDSKDSTYSMSSTLTLTKDEYERHNSYTCEATHKTSTSPIVKSFNRNEC

SEQ ID NO: 40 - protein, 663 aa, synthetic construct
QVQLQQSGPGLVQPSQSLSITCTVSGFSLTSYGIHWVRQSPGKGLEWLGVIWRGGGTDSNAAFMSRLSITKDNSKSQVFFKMNSLQADDTAIYYCARSRYDEEESMNYWGQGTSVTVSSASTKGPSVFPLAPSSKSTSGGTAALGCLVKDYFPEPVTVSWNSGALTSGVHTFPAVLQSSGLYSLSSVVTVPSSSLGTQTYICNVNHKPSNTKVDKKVEPKSCDKTHTCPPCPAPELLGGPSVFLFPPKPKDTLMISRTPEVTCVVVDVSHEDPEVKFNWYVDGVEVHNAKTKPREEQYNSTYRVVSVLTVLHQDWLNGKEYKCKVSNKALPAPIEKTISKAKGQPREPQVYTLPPSRDELTKNQVSLTCLVKGFYPSDIAVEWESNGQPENNYKTTPPVLDSDGSFFLYSKLTVDKSRWQQGNVFSCSVMHEALHNHYTQKSLSLSPGKQIVLTQSPASLSASVGETVTITCRASGNIHSYLAWYQQKQGKSPQLLVYNAKTLADGVPSRFSGSGSGTQYSLKINSLQPEDFGSYYCQHFWNTPPTFGAGTKLELKRTVAAPSVFIFPPSDEQLKSGTASVVCLLNNFYPREAKVQWKVDNALQSGNSQESVTEQDSKDSTYSLSSTLTLSKADYEKHKVYACEVTHQGLSSPVTKSFNRGEC

SEQ ID NO: 41 - protein, 663 aa, synthetic construct
QVQLQESGPGLVKPSETLSLTCTVSGFSLTSYGIHWIRQSPGRGLEWIGVIWRGGGTDSNAAFMSRITISRDTSKTQVSLKLGSVTAADTAIYYCARSRYDEEESMNYWGQGTSVTVSSASTKGPSVFPLAPSSKSTSGGTAALGCLVKDYFPEPVTVSWNSGALTSGVHTFPAVLQSSGLYSLSSVVTVPSSSLGTQTYICNVNHKPSNTKVDKKVEPKSCDKTHTCPPCPAPELLGGPSVFLFPPKPKDTLMISRTPEVTCVVVDVSHEDPEVKFNWYVDGVEVHNAKTKPREEQYNSTYRVVSVLTVLHQDWLNGKEYKCKVSNKALPAPIEKTISKAKGQPREPQVYTLPPSRDELTKNQVSLTCLVKGFYPSDIAVEWESNGQPENNYKTTPPVLDSDGSFFLYSKLTVDKSRWQQGNVFSCSVMHEALHNHYTQKSLSLSPGKEIVLTQSPSSLSASVGDSVTITCRASGNIHSYLAWYQQKPGKAPKLLIYNAKTLADGVPSRFSGSGSGTQYTLTISSLQPEDFATYYCQHFWNTPPTFGAGTKLELKRTVAAPSVFIFPPSDEQLKSGTASVVCLLNNFYPREAKVQWKVDNALQSGNSQESVTEQDSKDSTYSLSSTLTLSKADYEKHKVYACEVTHQGLSSPVTKSFNRGEC

SEQ ID NO: 42 - protein, 663 aa, synthetic construct
QVQLQESGPGLVKPSETLSLTCTVSGFSLTSYGIHWIRQSPGRGLEWIGVIWRGGGTDSNAAFMSRITISRDTSKTQVSLKLGSVTAADTAIYYCARSRYDEEESMNYWGQGTSVTVSSASTKGPSVFPLAPSSKSTSGGTAALGCLVKDYFPEPVTVSWNSGALTSGVHTFPAVLQSSGLYSLSSVVTVPSSSLGTQTYICNVNHKPSNTKVDKKVEPKSCDKTHTCPPCPAPELLGGPSVFLFPPKPKDTLMISRTPEVTCVVVDVSHEDPEVKFNWYVDGVEVHNAKTKPREEQYNSTYRVVSVLTVLHQDWLNGKEYKCKVSNKALPAPIEKTISKAKGQPREPQVYTLPPSRDELTKNQVSLTCLVKGFYPSDIAVEWESNGQPENNYKTTPPVLDSDGSFFLYSKLTVDKSRWQQGNVFSCSVMHEALHNHYTQKSLSLSPGKQIQLTQSPSFLSASVGDSVTITCRASGNIHSYLAWYQQKPGKAPQLLIYNAKTLADGVPSRFSGSGSGTEYTLTISSLQPEDFATYYCQHFWNTPPTFGAGTKLELKRTVAAPSVFIFPPSDEQLKSGTASVVCLLNNFYPREAKVQWKVDNALQSGNSQESVTEQDSKDSTYSLSSTLTLSKADYEKHKVYACEVTHQGLSSPVTKSFNRGEC

SEQ ID NO: 43 - protein, 663 aa, synthetic construct
QVQLQESGPGLVKPSETLSLTCTVSGFSLTSYGIHWIRQSPGRGLEWIGVIWRGGGTDSNAAFMSRITISRDTSKTQVSLKLGSVTAADTAIYYCARSRYDEEESMNYWGQGTSVTVSSASTKGPSVFPLAPSSKSTSGGTAALGCLVKDYFPEPVTVSWNSGALTSGVHTFPAVLQSSGLYSLSSVVTVPSSSLGTQTYICNVNHKPSNTKVDKKVEPKSCDKTHTCPPCPAPELLGGPSVFLFPPKPKDTLMISRTPEVTCVVVDVSHEDPEVKFNWYVDGVEVHNAKTKPREEQYNSTYRVVSVLTVLHQDWLNGKEYKCKVSNKALPAPIEKTISKAKGQPREPQVYTLPPSRDELTKNQVSLTCLVKGFYPSDIAVEWESNGQPENNYKTTPPVLDSDGSFFLYSKLTVDKSRWQQGNVFSCSVMHEALHNHYTQKSLSLSPGKEIVLTQSPATLSLSPGERATLSCRASGNIHSYLAWYQQKPGQAPRLLIYNAKTLADGIPARFSGSGSGTDYTLTISSLEPEDFASYYCQHFWNTPPTFGAGTKLELKRTVAAPSVFIFPPSDEQLKSGTASVVCLLNNFYPREAKVQWKVDNALQSGNSQESVTEQDSKDSTYSLSSTLTLSKADYEKHKVYACEVTHQGLSSPVTKSFNRGEC

SEQ ID NO: 44 - protein, 663 aa, synthetic construct
QVQLQESGPGLVKPSETLSLTCTVSGFSLTSYGIHWIRQSPGRGLEWIGVIWRGGGTDSNAAFMSRITISRDTSKTQVSLKLGSVTAADTAIYYCARSRYDEEESMNYWGQGTSVTVSSASTKGPSVFPLAPSSKSTSGGTAALGCLVKDYFPEPVTVSWNSGALTSGVHTFPAVLQSSGLYSLSSVVTVPSSSLGTQTYICNVNHKPSNTKVDKKVEPKSCDKTHTCPPCPAPELLGGPSVFLFPPKPKDTLMISRTPEVTCVVVDVSHEDPEVKFNWYVDGVEVHNAKTKPREEQYNSTYRVVSVLTVLHQDWLNGKEYKCKVSNKALPAPIEKTISKAKGQPREPQVYTLPPSRDELTKNQVSLTCLVKGFYPSDIAVEWESNGQPENNYKTTPPVLDSDGSFFLYSKLTVDKSRWQQGNVFSCSVMHEALHNHYTQKSLSLSPGKEIVLTQSPGTLSLSPGERATLSCRASGNIHSYLAWYQQKPGQAPRLLIYNAKTLADGIPDRFSGSGSGTDYTLTISRLEPEDFAVYYCQHFWNTPPTFGAGTKLELKRTVAAPSVFIFPPSDEQLKSGTASVVCLLNNFYPREAKVQWKVDNALQSGNSQESVTEQDSKDSTYSLSSTLTLSKADYEKHKVYACEVTHQGLSSPVTKSFNRGEC

SEQ ID NO: 45 - protein, 663 aa, synthetic construct; identical to SEQ ID NO: 41

SEQ ID NO: 46 - protein, 663 aa, synthetic construct; identical to SEQ ID NO: 42

SEQ ID NO: 47 - protein, 663 aa, synthetic construct; identical to SEQ ID NO: 43

SEQ ID NO: 48 - protein, 663 aa, synthetic construct; identical to SEQ ID NO: 44

SEQ ID NO: 49 - protein, 116 aa, Homo sapiens
EVQLVESGGGLVKPGGSLRLSCAASGFTFRSYSMNWVRQAPGKGLEWVSSIISSSSYIYYADSVKGRFTISRDNAKNSLYLQMNSLRAEDTALYYCARDQNAMDVWGQGTTVTVSS

SEQ ID NO: 50 - protein, 215 aa, Homo sapiens
SYELTQPPSVSVAPGKTARITCAGNNIGSKSVHWYQQKPGQAPVLVIYYDSDRPSGIPERFSGSNSGNTATLTISRVEAGDEADYYCQVWDSGSDHPWVFGGGTKLTVLRQPKAAPSVTLFPPSSEELQANKATLVCLISDFYPGAVTVAWKADSSPVKAGVETTTPSKQSNNKYAASSYLSLTPEQWKSHRSYSCQVTHEGSTVEKTVAPTECS

SEQ ID NO: 51 - protein, 569 aa, Homo sapiens
EVQLVESGGGLVKPGGSLRLSCAASGFTFSGYSMNWVRQAPGKGLEWVSSISSSSTYIYYVDSVRGRFTISRDNAKNSLYLQMNSLRAEDTAVYYCARDENDMDVWGQGTTVTVSSGSASAPTLFPLVSCENSPSDTSSVAVGCLAQDFLPDSITFSWKYKNNSDISSTRGFPSVLRGGKYAATSQVLLPSKDVMQGTDEHVVCKVQHPNGNKEKNVPLPVIAELPPKVSVFVPPRDGFFGNPRKSKLICQATGFSPRQIQVSWLREGKQVGSGVTTDQVQAEAKESGPTTYKVTSTLTIKESDWLSQSMFTCRVDHRGLTFQQNASSMCVPDQDTAIRVFAIPPSFASIFLTKSTKLTCLVTDLTTYDSVTISWTRQNGEAVKTHTNISESHPNATFSAVGEASICEDDWNSGERFTCTVTHTDLPSPLKQTISRPKGVALHRPDVYLLPPAREQLNLRESATITCLVTGFSPADVFVQWMQRGQPLSPEKYVTSAPMPEPQAPGRYFAHSILTVSEEEWNTGETYTCVVAHEALPNRVTERTVDKSTGKPTLYNVSLVMSDTAGTCY

SEQ ID NO: 52 - protein, 215 aa, Homo sapiens
SYVLTQPPSVSVAPGKTARITCGGNNIGTKSVHWYQQKPGQAPVLVIYYDSDRPSGIPERFSGSNSGNTATLTISRVEAGDEADYYCQVWDSGSDHPWVFGGGTKLTVLRQPKAAPSVTLFPPSSEELQANKATLVCLISDFYPGAVTVAWKADSSPVKAGVETTTPSKQSNNKYAASSYLSLTPEQWKSHRSYSCQVTHEGSTVEKTVAPTECS

SEQ ID NO: 53 - protein, 110 aa, Homo sapiens
SYELTQPPSVSVAPGKTARITCAGNNIGSKSVHWYQQKPGQAPVLVIYYDSDRPSGIPERFSGSNSGNTATLTISRVEAGDEADYYCQVWDSGSDHPWVFGGGTKLTVLR